European Patent Application EP 4 516 802 A1, published March 5, 2025. Title: 신규 염증해소 펩타이드 및 그의 용도. Applicant: (주)노바셀테크놀로지. The sequence listing filed with the application follows.

SEQUENCE LISTING (160 sequences)

SEQ ID NO: 1 - protein, 7 aa, synthetic construct
  VARIANT 7: note = X is D-type methionine
RWRYKVX

SEQ ID NO: 2 - protein, 7 aa, synthetic construct
  VARIANT 7: note = X is D-type methionine
  VARIANT <1: note = The N-terminus is modified with an octanoyl group.
RWRYKVX

SEQ ID NO: 3 - protein, 6 aa, synthetic construct
  VARIANT 6: note = X is D-type methionine
WRYKVX

SEQ ID NO: 4 - protein, 7 aa, synthetic construct
  VARIANT 7: note = X is D-type methionine
  VARIANT <1: note = The N-terminus is modified with an acetyl group
KWKYKVX

SEQ ID NO: 5 - protein, 7 aa, synthetic construct
  VARIANT 7: note = X is D-type methionine
RMRYKVX

SEQ ID NO: 6 - protein, 7 aa, synthetic construct
  VARIANT 7: note = X is D-type methionine
  VARIANT <1: note = The N-terminus is modified with an acetyl group
RMRYKVX

SEQ ID NO: 7 - protein, 7 aa, synthetic construct
  VARIANT 7: note = X is D-type methionine
  VARIANT <1: note = The N-terminus is modified with a butanoyl group.
RMRYKVX

SEQ ID NO: 8 - protein, 7 aa, synthetic construct
  VARIANT 7: note = X is D-type methionine
  VARIANT <1: note = The N-terminus is modified with an octanoyl group.
RMRYKVX

SEQ ID NO: 9 - protein, 7 aa, synthetic construct
  VARIANT 7: note = X is D-type methionine
KMKYKVX

SEQ ID NO: 10 - protein, 7 aa, synthetic construct
  VARIANT 7: note = X is D-type methionine
  VARIANT <1: note = The N-terminus is modified with an acetyl group
KMKYKVX

SEQ ID NO: 11 - protein, 7 aa, synthetic construct
  VARIANT 7: note = X is D-type methionine
  VARIANT <1: note = The N-terminus is modified with a butanoyl group.
KMKYKVX

SEQ ID NO: 12 - protein, 7 aa, synthetic construct
  VARIANT 7: note = X is D-type methionine
  VARIANT <1: note = The N-terminus is modified with an octanoyl group.
KMKYKVX

SEQ ID NO: 13 - protein, 6 aa, synthetic construct
  VARIANT 6: note = X is D-type methionine
MRYKVX

SEQ ID NO: 14 - protein, 6 aa, synthetic construct
  VARIANT 6: note = X is D-type methionine
  VARIANT <1: note = The N-terminus is modified with an acetyl group
MRYKVX

SEQ ID NO: 15 - protein, 6 aa, synthetic construct
  VARIANT 6: note = X is D-type methionine
  VARIANT <1: note = The N-terminus is modified with a butanoyl group.
MRYKVX

SEQ ID NO: 16 - protein, 6 aa, synthetic construct
  VARIANT 6: note = X is D-type methionine
  VARIANT <1: note = The N-terminus is modified with an octanoyl group.
MRYKVX

SEQ ID NO: 17 - protein, 6 aa, synthetic construct
  VARIANT 6: note = X is D-type methionine
MKYKVX

SEQ ID NO: 18 - protein, 6 aa, synthetic construct
  VARIANT 6: note = X is D-type methionine
  VARIANT <1: note = The N-terminus is modified with an acetyl group
MKYKVX

SEQ ID NO: 19 - protein, 6 aa, synthetic construct
  VARIANT 6: note = X is D-type methionine
  VARIANT <1: note = The N-terminus is modified with a butanoyl group.
MKYKVX

SEQ ID NO: 20 - protein, 6 aa, synthetic construct
  VARIANT 6: note = X is D-type methionine
  VARIANT <1: note = The N-terminus is modified with an octanoyl group.
MKYKVX

SEQ ID NO: 21 - protein, 7 aa, synthetic construct
  VARIANT 7: note = X is D-type methionine
HMKYKVX

SEQ ID NO: 22 - protein, 7 aa, synthetic construct
  VARIANT 7: note = X is D-type methionine
  VARIANT <1: note = The N-terminus is modified with an acetyl group.
HMKYKVX

SEQ ID NO: 23 - protein, 7 aa, synthetic construct
  VARIANT 7: note = X is D-type methionine
  VARIANT <1: note = The N-terminus is modified with a butanoyl group.
HMKYKVX

SEQ ID NO: 24 - protein, 7 aa, synthetic construct
  VARIANT 7: note = X is D-type methionine
  VARIANT <1: note = The N-terminus is modified with an octanoyl group.
HMKYKVX

SEQ ID NO: 25 - protein, 7 aa, synthetic construct
  VARIANT 7: note = X is D-type methionine
PMKYKVX

SEQ ID NO: 26 - protein, 7 aa, synthetic construct
  VARIANT 7: note = X is D-type methionine
  VARIANT <1: note = The N-terminus is modified with an acetyl group.
PMKYKVX

SEQ ID NO: 27 - protein, 7 aa, synthetic construct
  VARIANT 7: note = X is D-type methionine
  VARIANT <1: note = The N-terminus is modified with a butanoyl group.
PMKYKVX

SEQ ID NO: 28 - protein, 7 aa, synthetic construct
  VARIANT 7: note = X is D-type methionine
  VARIANT <1: note = The N-terminus is modified with an octanoyl group.
PMKYKVX

SEQ ID NO: 29 - protein, 7 aa, synthetic construct
  VARIANT 7: note = X is D-type methionine
RWRYRVX

SEQ ID NO: 30 - protein, 7 aa, synthetic construct
  VARIANT 7: note = X is D-type methionine
RMRYRVX

SEQ ID NO: 31 - protein, 7 aa, synthetic construct
  VARIANT 7: note = X is D-type methionine
HMRYRVX

SEQ ID NO: 32 - protein, 7 aa, synthetic construct
  VARIANT 7: note = X is D-type methionine
RWRYKYX

SEQ ID NO: 33 - protein, 7 aa, synthetic construct
  VARIANT 7: note = X is D-type methionine
  VARIANT <1: note = The N-terminus is modified with an acetyl group.
RWRYKYX

SEQ ID NO: 34 - protein, 7 aa, synthetic construct
  VARIANT 7: note = X is D-type methionine
  VARIANT <1: note = The N-terminus is modified with an octanoyl group.
RWRYKYX

SEQ ID NO: 35 - protein, 6 aa, synthetic construct
  VARIANT 6: note = X is D-type methionine
WRYKYX

SEQ ID NO: 36 - protein, 7 aa, synthetic construct
  VARIANT 7: note = X is D-type methionine
  VARIANT <1: note = The N-terminus is modified with an acetyl group.
KWKYKYX

SEQ ID NO: 37 - protein, 7 aa, synthetic construct
  VARIANT 7: note = X is D-type methionine
  VARIANT <1: note = The N-terminus is modified with a butanoyl group.
HWKYKYX

SEQ ID NO: 38 - protein, 7 aa, synthetic construct
  VARIANT 7: note = X is D-type methionine
RMRYKYX

SEQ ID NO: 39 - protein, 7 aa, synthetic construct
  VARIANT 7: note = X is D-type methionine
  VARIANT <1: note = The N-terminus is modified with an acetyl group.
RMRYKYX

SEQ ID NO: 40 - protein, 7 aa, synthetic construct
  VARIANT 7: note = X is D-type methionine
  VARIANT <1: note = The N-terminus is modified with an octanoyl group.
RMRYKYX

SEQ ID NO: 41 - protein, 6 aa, synthetic construct
  VARIANT 6: note = X is D-type methionine
MRYKYX

SEQ ID NO: 42 - protein, 6 aa, synthetic construct
  VARIANT 6: note = X is D-type methionine
  VARIANT <1: note = The N-terminus is modified with an acetyl group.
MRYKYX

SEQ ID NO: 43 - protein, 6 aa, synthetic construct
  VARIANT 6: note = X is D-type methionine
  VARIANT <1: note = The N-terminus is modified with a butanoyl group.
MRYKYX

SEQ ID NO: 44 - protein, 7 aa, synthetic construct
  VARIANT 7: note = X is D-type methionine
HMRYKYX

SEQ ID NO: 45 - protein, 7 aa, synthetic construct
  VARIANT 7: note = X is D-type methionine
  VARIANT <1: note = The N-terminus is modified with a butanoyl group.
HMRYKYX

SEQ ID NO: 46 - protein, 7 aa, synthetic construct
  VARIANT 7: note = X is D-type methionine
PMRYKYX

SEQ ID NO: 47 - protein, 7 aa, synthetic construct
  VARIANT 7: note = X is D-type methionine
  VARIANT <1: note = The N-terminus is modified with a butanoyl group.
PMRYKYX

SEQ ID NO: 48 - protein, 7 aa, synthetic construct
  VARIANT 7: note = X is D-type methionine
RWRYRYX

SEQ ID NO: 49 - protein, 6 aa, synthetic construct
  VARIANT 6: note = X is D-type methionine
  VARIANT <1: note = The N-terminus is modified with an acetyl group.
MRYRYX

SEQ ID NO: 50 - protein, 7 aa, synthetic construct
  VARIANT 7: note = X is D-type methionine
RMRYKPX

SEQ ID NO: 51 - protein, 7 aa, synthetic construct
  VARIANT 7: note = X is D-type methionine
  VARIANT <1: note = The N-terminus is modified with an acetyl group.
RMRYKPX

SEQ ID NO: 52 - protein, 7 aa, synthetic construct
  VARIANT 7: note = X is D-type methionine
  VARIANT <1: note = The N-terminus is modified with a butanoyl group.
RMRYKPX

SEQ ID NO: 53 - protein, 7 aa, synthetic construct
  VARIANT 7: note = X is D-type methionine
  VARIANT <1: note = The N-terminus is modified with an octanoyl group.
RMRYKPX

SEQ ID NO: 54 - protein, 6 aa, synthetic construct
  VARIANT 6: note = X is D-type methionine
MRYKPX

SEQ ID NO: 55 - protein, 6 aa, synthetic construct
  VARIANT 6: note = X is D-type methionine
  VARIANT <1: note = The N-terminus is modified with an acetyl group.
MRYKPX

SEQ ID NO: 56 - protein, 6 aa, synthetic construct
  VARIANT 6: note = X is D-type methionine
  VARIANT <1: note = The N-terminus is modified with a butanoyl group.
MRYKPX

SEQ ID NO: 57 - protein, 6 aa, synthetic construct
  VARIANT 6: note = X is D-type methionine
  VARIANT <1: note = The N-terminus is modified with an octanoyl group.
MRYKPX

SEQ ID NO: 58 - protein, 7 aa, synthetic construct
  VARIANT 7: note = X is D-type methionine
HMRYKPX

SEQ ID NO: 59 - protein, 7 aa, synthetic construct
  VARIANT 7: note = X is D-type methionine
  VARIANT <1: note = The N-terminus is modified with an acetyl group.
HMRYKPX

SEQ ID NO: 60 - protein, 7 aa, synthetic construct
  VARIANT 7: note = X is D-type methionine
  VARIANT <1: note = The N-terminus is modified with a butanoyl group.
HMRYKPX

SEQ ID NO: 61 - protein, 7 aa, synthetic construct
  VARIANT 7: note = X is D-type methionine
  VARIANT <1: note = The N-terminus is modified with an octanoyl group.
HMRYKPX

SEQ ID NO: 62 - protein, 7 aa, synthetic construct
  VARIANT 7: note = X is D-type methionine
PMRYKPX

SEQ ID NO: 63 - protein, 7 aa, synthetic construct
  VARIANT 7: note = X is D-type methionine
  VARIANT <1: note = The N-terminus is modified with an acetyl group.
PMRYKPX

SEQ ID NO: 64 - protein, 7 aa, synthetic construct
  VARIANT 7: note = X is D-type methionine
  VARIANT <1: note = The N-terminus is modified with a butanoyl group.
PMRYKPX

SEQ ID NO: 65 - protein, 7 aa, synthetic construct
  VARIANT 7: note = X is D-type methionine
  VARIANT <1: note = The N-terminus is modified with an octanoyl group.
PMRYKPX

SEQ ID NO: 66 - protein, 7 aa, synthetic construct
  VARIANT 7: note = X is D-type methionine
KMKYKPX

SEQ ID NO: 67 - protein, 7 aa, synthetic construct
  VARIANT 7: note = X is D-type methionine
  VARIANT <1: note = The N-terminus is modified with an acetyl group.
KMKYKPX

SEQ ID NO: 68 - protein, 7 aa, synthetic construct
  VARIANT 7: note = X is D-type methionine
  VARIANT <1: note = The N-terminus is modified with a butanoyl group.
KMKYKPX

SEQ ID NO: 69 - protein, 7 aa, synthetic construct
  VARIANT 7: note = X is D-type methionine
  VARIANT <1: note = The N-terminus is modified with an octanoyl group.
KMKYKPX

SEQ ID NO: 70 - protein, 6 aa, synthetic construct
  VARIANT 6: note = X is D-type methionine
MKYKPX

SEQ ID NO: 71 - protein, 6 aa, synthetic construct
  VARIANT 6: note = X is D-type methionine
  VARIANT <1: note = The N-terminus is modified with an acetyl group.
MKYKPX

SEQ ID NO: 72 - protein, 6 aa, synthetic construct
  VARIANT 6: note = X is D-type methionine
  VARIANT <1: note = The N-terminus is modified with a butanoyl group.
MKYKPX

SEQ ID NO: 73 - protein, 6 aa, synthetic construct
  VARIANT 6: note = X is D-type methionine
  VARIANT <1: note = The N-terminus is modified with an octanoyl group.
MKYKPX

SEQ ID NO: 74 - protein, 7 aa, synthetic construct
  VARIANT 7: note = X is D-type methionine
RWRYKPX

SEQ ID NO: 75 - protein, 7 aa, synthetic construct
  VARIANT 7: note = X is D-type methionine
  VARIANT <1: note = The N-terminus is modified with a butanoyl group.
RWRYKPX

SEQ ID NO: 76 - protein, 6 aa, synthetic construct
  VARIANT 6: note = X is D-type methionine
  VARIANT <1: note = The N-terminus is modified with an acetyl group.
WRYKPX

SEQ ID NO: 77 - protein, 7 aa, synthetic construct
  VARIANT 7: note = X is D-type methionine
RWRYWYX

SEQ ID NO: 78 - protein, 7 aa, synthetic construct
  VARIANT 7: note = X is D-type methionine
  VARIANT <1: note = The N-terminus is modified with an acetyl group.
RWRYWYX

SEQ ID NO: 79 - protein, 6 aa, synthetic construct
  VARIANT 6: note = X is D-type methionine
WRYWYX

SEQ ID NO: 80 - protein, 7 aa, synthetic construct
  VARIANT 7: note = X is D-type methionine
  VARIANT <1: note = The N-terminus is modified with an acetyl group.
KWKYWYX

SEQ ID NO: 81 - protein, 7 aa, synthetic construct
  VARIANT 7: note = X is D-type methionine
RMRYWYX

SEQ ID NO: 82 - protein, 7 aa, synthetic construct
  VARIANT 7: note = X is D-type methionine
  VARIANT <1: note = The N-terminus is modified with an acetyl group.
RMRYWYX

SEQ ID NO: 83 - protein, 7 aa, synthetic construct
  VARIANT 7: note = X is D-type methionine
  VARIANT <1: note = The N-terminus is modified with a butanoyl group.
RMRYWYX

SEQ ID NO: 84 - protein, 7 aa, synthetic construct
  VARIANT 7: note = X is D-type methionine
  VARIANT <1: note = The N-terminus is modified with an octanoyl group.
RMRYWYX

SEQ ID NO: 85 - protein, 6 aa, synthetic construct
  VARIANT 6: note = X is D-type methionine
MRYWYX

SEQ ID NO: 86 - protein, 6 aa, synthetic construct
  VARIANT 6: note = X is D-type methionine
  VARIANT <1: note = The N-terminus is modified with an acetyl group.
MRYWYX

SEQ ID NO: 87 - protein, 6 aa, synthetic construct
  VARIANT 6: note = X is D-type methionine
  VARIANT <1: note = The N-terminus is modified with a butanoyl group.
MRYWYX

SEQ ID NO: 88 - protein, 6 aa, synthetic construct
  VARIANT 6: note = X is D-type methionine
  VARIANT <1: note = The N-terminus is modified with an octanoyl group.
MRYWYX

SEQ ID NO: 89 - protein, 6 aa, synthetic construct
  VARIANT 6: note = X is D-type methionine
MKYWYX

SEQ ID NO: 90 - protein, 6 aa, synthetic construct
  VARIANT 6: note = X is D-type methionine
  VARIANT <1: note = The N-terminus is modified with an acetyl group.
MKYWYX

SEQ ID NO: 91 - protein, 6 aa, synthetic construct
  VARIANT 6: note = X is D-type methionine
  VARIANT <1: note = The N-terminus is modified with a butanoyl group.
MKYWYX

SEQ ID NO: 92 - protein, 7 aa, synthetic construct
  VARIANT 7: note = X is D-type methionine
  VARIANT <1: note = The N-terminus is modified with an acetyl group.
HMRYWYX

SEQ ID NO: 93 - protein, 7 aa, synthetic construct
  VARIANT 7: note = X is D-type methionine
  VARIANT <1: note = The N-terminus is modified with a butanoyl group.
HMRYWYX

SEQ ID NO: 94 - protein, 7 aa, synthetic construct
  VARIANT 7: note = X is D-type methionine
RWRYYVX

SEQ ID NO: 95 - protein, 6 aa, synthetic construct
  VARIANT 6: note = X is D-type methionine
  VARIANT <1: note = The N-terminus is modified with an acetyl group.
WRYYVX

SEQ ID NO: 96 - protein, 7 aa, synthetic construct
  VARIANT 7: note = X is D-type methionine
KWKYYVX

SEQ ID NO: 97 - protein, 7 aa, synthetic construct
  VARIANT 7: note = X is D-type methionine
RMRYYVX

SEQ ID NO: 98 - protein, 7 aa, synthetic construct
  VARIANT 7: note = X is D-type methionine
  VARIANT <1: note = The N-terminus is modified with an acetyl group.
RMRYYVX

SEQ ID NO: 99 - protein, 7 aa, synthetic construct
  VARIANT 7: note = X is D-type methionine
  VARIANT <1: note = The N-terminus is modified with an octanoyl group.
RMRYYVX

SEQ ID NO: 100 - protein, 6 aa, synthetic construct
  VARIANT 6: note = X is D-type methionine
MRYYVX

SEQ ID NO: 101 - protein, 7 aa, synthetic construct
  VARIANT 7: note = X is D-type methionine
RWRYWVX

SEQ ID NO: 102 - protein, 6 aa, synthetic construct
  VARIANT 6: note = X is D-type methionine
  VARIANT <1: note = The N-terminus is modified with an acetyl group.
WRYWVX

SEQ ID NO: 103 - protein, 7 aa, synthetic construct
  VARIANT 7: note = X is D-type methionine
  VARIANT <1: note = The N-terminus is modified with an acetyl group.
KWKYWVX

SEQ ID NO: 104 - protein, 7 aa, synthetic construct
  VARIANT 7: note = X is D-type methionine
  VARIANT <1: note = The N-terminus is modified with an acetyl group.
RMRYWVX

SEQ ID NO: 105 - protein, 6 aa, synthetic construct
  VARIANT 6: note = X is D-type methionine
  VARIANT <1: note = The N-terminus is modified with an acetyl group.
MRYWVX

SEQ ID NO: 106 - protein, 7 aa, synthetic construct
  VARIANT 7: note = X is D-type methionine
RMRYWPX

SEQ ID NO: 107 - protein, 7 aa, synthetic construct
  VARIANT 7: note = X is D-type methionine
  VARIANT <1: note = The N-terminus is modified with an acetyl group.
RMRYWPX

SEQ ID NO: 108 - protein, 7 aa, synthetic construct
  VARIANT 7: note = X is D-type methionine
  VARIANT <1: note = The N-terminus is modified with a butanoyl group.
RMRYWPX

SEQ ID NO: 109 - protein, 7 aa, synthetic construct
  VARIANT 7: note = X is D-type methionine
  VARIANT <1: note = The N-terminus is modified with an octanoyl group.
RMRYWPX

SEQ ID NO: 110 - protein, 6 aa, synthetic construct
  VARIANT 6: note = X is D-type methionine
MRYWPX

SEQ ID NO: 111 - protein, 6 aa, synthetic construct
  VARIANT 6: note = X is D-type methionine
  VARIANT <1: note = The N-terminus is modified with an acetyl group.
MRYWPX

SEQ ID NO: 112 - protein, 6 aa, synthetic construct
  VARIANT 6: note = X is D-type methionine
  VARIANT <1: note = The N-terminus is modified with a butanoyl group.
MRYWPX

SEQ ID NO: 113 - protein, 6 aa, synthetic construct
  VARIANT 6: note = X is D-type methionine
MKYWPX

SEQ ID NO: 114 - protein, 6 aa, synthetic construct
  VARIANT 6: note = X is D-type methionine
  VARIANT <1: note = The N-terminus is modified with an acetyl group.
MKYWPX

SEQ ID NO: 115 - protein, 6 aa, synthetic construct
  VARIANT 6: note = X is D-type methionine
  VARIANT <1: note = The N-terminus is modified with a butanoyl group.
MKYWPX

SEQ ID NO: 116 - protein, 6 aa, synthetic construct
  VARIANT 6: note = X is D-type methionine
  VARIANT <1: note = The N-terminus is modified with an octanoyl group.
MKYWPX

SEQ ID NO: 117 - protein, 7 aa, synthetic construct
  VARIANT 7: note = X is D-type methionine
  VARIANT <1: note = The N-terminus is modified with an acetyl group.
RWRYWPX

SEQ ID NO: 118 - protein, 6 aa, synthetic construct
  VARIANT 6: note = X is D-type methionine
WRYWPX

SEQ ID NO: 119 - protein, 7 aa, synthetic construct
  VARIANT 7: note = X is D-type methionine
  VARIANT <1: note = The N-terminus is modified with an acetyl group.
RMRYYPX

SEQ ID NO: 120 - protein, 6 aa, synthetic construct
  VARIANT 6: note = X is D-type methionine
MRYYPX

SEQ ID NO: 121 - protein, 7 aa, synthetic construct
  VARIANT 7: note = X is D-type methionine
  VARIANT <1: note = The N-terminus is modified with an acetyl group.
RWRYYPX

SEQ ID NO: 122 - protein, 6 aa, synthetic construct
  VARIANT 6: note = X is D-type methionine
  VARIANT <1: note = The N-terminus is modified with an acetyl group.
WRYYPX

SEQ ID NO: 123 - protein, 7 aa, synthetic construct
  VARIANT 7: note = X is D-type methionine
RWRYYYX

SEQ ID NO: 124 - protein, 6 aa, synthetic construct
  VARIANT 6: note = X is D-type methionine
  VARIANT <1: note = The N-terminus is modified with an acetyl group.
WRYYYX

SEQ ID NO: 125 - protein, 7 aa, synthetic construct
  VARIANT 7: note = X is D-type methionine
  VARIANT <1: note = The N-terminus is modified with an acetyl group.
RMRYYYX

SEQ ID NO: 126 - protein, 6 aa, synthetic construct
  VARIANT 6: note = X is D-type methionine
MRYYYX

SEQ ID NO: 127 - protein, 7 aa, synthetic construct
  VARIANT 7: note = X is D-type methionine
  VARIANT <1: note = The N-terminus is modified with a butanoyl group.
HMKYYYX

SEQ ID NO: 128 - protein, 6 aa, synthetic construct
  VARIANT 6: note = X is D-type methionine
IKFWYX

SEQ ID NO: 129 - protein, 6 aa, synthetic construct
  VARIANT 6: note = X is D-type methionine
IKFWMX

SEQ ID NO: 130 - protein, 6 aa, synthetic construct
  VARIANT 6: note = X is D-type methionine
IKKWMX

SEQ ID NO: 131 - protein, 6 aa, synthetic construct
  VARIANT 6: note = X is D-type methionine
IKFKYX

SEQ ID NO: 132 - protein, 6 aa, synthetic construct
  VARIANT 6: note = X is D-type methionine
IKFKVX

SEQ ID NO: 133 - protein, 6 aa, synthetic construct
  VARIANT 6: note = X is D-type methionine
IKFKPX

SEQ ID NO: 134 - protein, 6 aa, synthetic construct
  VARIANT 6: note = X is D-type methionine
IKYKVX

SEQ ID NO: 135 - protein, 6 aa, synthetic construct
  VARIANT 6: note = X is D-type methionine
  VARIANT <1: note = The N-terminus is modified with an acetyl group.
IKYKVX

SEQ ID NO: 136 - protein, 6 aa, synthetic construct
  VARIANT 6: note = X is D-type methionine
  VARIANT <1: note = The N-terminus is modified with a butanoyl group.
IKYKVX

SEQ ID NO: 137 - protein, 6 aa, synthetic construct
  VARIANT 6: note = X is D-type methionine
  VARIANT <1: note = The N-terminus is modified with an octanoyl group.
IKYKVX

SEQ ID NO: 138 - protein, 6 aa, synthetic construct
  VARIANT 6: note = X is D-type methionine
PKYKVX

SEQ ID NO: 139 - protein, 6 aa, synthetic construct
  VARIANT 6: note = X is D-type methionine
  VARIANT <1: note = The N-terminus is modified with an acetyl group.
PKYKVX

SEQ ID NO: 140 - protein, 6 aa, synthetic construct
  VARIANT 6: note = X is D-type methionine
  VARIANT <1: note = The N-terminus is modified with a butanoyl group.
PKYKVX

SEQ ID NO: 141 - protein, 6 aa, synthetic construct
  VARIANT 6: note = X is D-type methionine
  VARIANT <1: note = The N-terminus is modified with an octanoyl group.
PKYKVX

SEQ ID NO: 142 - protein, 6 aa, synthetic construct
  VARIANT 6: note = X is D-type methionine
IKYKPX

SEQ ID NO: 143 - protein, 6 aa, synthetic construct
  VARIANT 6: note = X is D-type methionine
  VARIANT <1: note = The N-terminus is modified with an acetyl group.
IKYKPX

SEQ ID NO: 144 - protein, 6 aa, synthetic construct
  VARIANT 6: note = X is D-type methionine
  VARIANT <1: note = The N-terminus is modified with a butanoyl group.
IKYKPX

SEQ ID NO: 145 - protein, 6 aa, synthetic construct
  VARIANT 6: note = X is D-type methionine
  VARIANT <1: note = The N-terminus is modified with an octanoyl group.
IKYKPX

SEQ ID NO: 146 - protein, 6 aa, synthetic construct
  VARIANT 6: note = X is D-type methionine
HKYKPX

SEQ ID NO: 147 - protein, 6 aa, synthetic construct
  VARIANT 6: note = X is D-type methionine
  VARIANT <1: note = The N-terminus is modified with an acetyl group.
HKYKPX

SEQ ID NO: 148 - protein, 6 aa, synthetic construct
  VARIANT 6: note = X is D-type methionine
  VARIANT <1: note = The N-terminus is modified with a butanoyl group.
HKYKPX

SEQ ID NO: 149 - protein, 6 aa, synthetic construct
  VARIANT 6: note = X is D-type methionine
  VARIANT <1: note = The N-terminus is modified with an octanoyl group.
HKYKPX

SEQ ID NO: 150 - protein, 6 aa, synthetic construct
  VARIANT 6: note = X is D-type methionine
  VARIANT <1: note = The N-terminus is modified with an acetyl group.
HKYWPX

SEQ ID NO: 151 - protein, 6 aa, synthetic construct
  VARIANT 6: note = X is D-type methionine
  VARIANT <1: note = The N-terminus is modified with a butanoyl group.
HKYWPX

SEQ ID NO: 152 - protein, 7 aa, synthetic construct
  VARIANT 7: note = X is D-type methionine
RWRYRIX

SEQ ID NO: 153 - protein, 7 aa, synthetic construct
  VARIANT 7: note = X is D-type methionine
RWRYRTX

SEQ ID NO: 154 - protein, 7 aa, synthetic construct
  VARIANT 7: note = X is D-type methionine
RWRYLYX

SEQ ID NO: 155 - protein, 7 aa, synthetic construct
  VARIANT 7: note = X is D-type methionine
RWRYNYX

SEQ ID NO: 156 - protein, 7 aa, synthetic construct
  VARIANT 7: note = X is D-type methionine
RWRYFYX

SEQ ID NO: 157 - protein, 7 aa, synthetic construct
  VARIANT 7: note = X is D-type methionine
RWRYTYX

SEQ ID NO: 158 - protein, 7 aa, synthetic construct
  VARIANT 7: note = X is D-type methionine
RWRYLVX

SEQ ID NO: 159 - protein, 7 aa, synthetic construct
  VARIANT 7: note = X is D-type methionine
RWRYNVX

SEQ ID NO: 160 - protein, 7 aa, synthetic construct
  VARIANT 7: note = X is D-type methionine
RWRYFVX